European Patent Specification EP 3 852 804 B1, published July 15, 2026. Title: Suppressing IgE-Mediated Allergy by Desensitization with Monovalent Anti-FCeRIa Monoclonal Antibody. Applicant: University of Cincinnati. The sequence listing filed with the application follows.

SEQUENCE LISTING (13 sequences)

SEQ ID NO: 1 - DNA, 324 bp, Homo sapiens
gatatcgtgatgacccaaactccatcttccatgtatgcatctctaggagagagagtcactatcacttgcaaggcgagtcaggacattaataactatttaagctggttccagcagaaaccagggagatctcctaagaccctgatctatcgtgcaaacagattgatggatggggtcccatcaaggatcagaggcagtggatctgggcaagattattctctcaccatcagcagcctggagtatgaagatatgggaatttattattgtctactatataatgagtttccgtggatgttcggtggaggcaccaagctggaaatcaaacgg

SEQ ID NO: 2 - DNA, 351 bp, Homo sapiens
caggtgcagctgcaggagtcagggggagacgtagtgaagcctggagggtccctgaaactctcctgtgcagcctctggattcactttcagtttctatggcatgtcttgggttcgtcagactccagacaagaaactggagtgggtcgcaaccattagtggtggtggtaattacacctactatccagacagtgtgaaggggcgattcaccatctccagagacaatgccatgaacaccctttacctgcaaatgaacagtctgaagtctgaagacacagccatgtattattgtgtgagagcctactatggtaattggaattcttactggggccaagggactctggtcactgtctct

SEQ ID NO: 3 - protein, 108 aa, Homo sapiens
DIVMTQTPSSMYASLGERVTITCKASQDINNYLSWFQQKPGRSPKTLIYRANRLMDGVPSRIRGSGSGQDYSLTISSLEYEDMGIYYCLLYNEFPWMFGGGTKLEIKR

SEQ ID NO: 4 - protein, 117 aa, Homo sapiens
QVQLQESGGDVVKPGGSLKLSCAASGFTFSFYGMSWVRQTPDKKLEWVATISGGGNYTYYPDSVKGRFTISRDNAMNTLYLQMNSLKSEDTAMYYCVRAYYGNWNSYWGQGTLVTVS

SEQ ID NO: 5 - protein, 6 aa, Homo sapiens
QDINNY

SEQ ID NO: 6 - protein, 3 aa, Homo sapiens
RAN

SEQ ID NO: 7 - protein, 9 aa, Homo sapiens
LLYNEFPWM

SEQ ID NO: 8 - protein, 8 aa, Homo sapiens
GFTFSFYG

SEQ ID NO: 9 - protein, 8 aa, Homo sapiens
ISGGGNYT

SEQ ID NO: 10 - protein, 11 aa, Homo sapiens
VRAYYGNWNSY

SEQ ID NO: 11 - protein, 234 aa, Homo sapiens
MYRMQLLSCIALSLALVTNSDIVMTQTPSSMYASLGERVTITCKASQDINNYLSWFQQKPGRSPKTLIYRANRLMDGVPSRIRGSGSGQDYSLTISSLEYEDMGIYYCLLYNEFPWMFGGGTKLEIKRTVAAPSVFIFPPSDEQLKSGTASVVCLLNNFYPREAKVQWKVDNALQSGNSQESVTEQDSKDSTYSLSSTLTLSKADYEKHKVYACEVTHQGLSSPVTKSFNRGEC

SEQ ID NO: 12 - protein, 469 aa, Homo sapiens
MYRMQLLSCIALSLALVTNSISQVQLQESGGDVVKPGGSLKLSCAASGFTFSFYGMSWVRQTPDKKLEWVATISGGGNYTYYPDSVKGRFTISRDNAMNTLYLQMNSLKSEDTAMYYCVRAYYGNWNSYWGQGTLVTVSASTKGPSVFPLAPSSKSTSGGTAALGCLVKDYFPEPVTVSWNSGALTSGVHTFPAVLQSSGLYSLSSVVTVPSSSLGTQTYICNVNHKPSNTKVDKKVEPKSCDKTHTCPPCPAPELLGGPSVFLFPPKPKDTLMISRTPEVTCVVVDVSHEDPEVKFNWYVDGVEVHNAKTKPREEQYNSTYRVVSVLTVLHQDWLNGKEYKCKVSNKALPAPIEKTISKAKGQPREPQVYTLPPSREEMTKNQVSLTCLVKGFYPSDIAVEWESNGQPENNYKTTPPVLDSDGSFFLYSKLTVDKSRWQQGNVFSCSVMHEALHNHYTQKSLSLSPGK

SEQ ID NO: 13 - protein, 247 aa, Homo sapiens
METDTLLLWVLLLWVPGSTGDKTHTCPPCPAPELLGGPSVFLFPPKPKDTLMISRTPEVTCVVVDVSHEDPEVKFNWYVDGVEVHNAKTKPREEQYNSTYRVVSVLTVLHQDWLNGKEYKCKVSNKALPAPIEKTISKAKGQPREPQVYTLPPSREEMTKNQVSLTCLVKGFYPSDIAVEWESNGQPENNYDTTPPVLDSDGSFFLYSDLTVDKSRWQQGNVFSCSVMHEALHNHYTQKSLSLSPGK